European Patent Specification EP 3 630 967 B1, published June 12, 2024. Title: Protease and binding polypeptide for O-glycoproteins. Applicant: GENOVIS AB. The sequence listing filed with the application follows.

SEQUENCE LISTING (50 sequences)

SEQ ID NO: 1 - protein, 361 aa, Akkermansia muciniphila
EVTVPDALKDRIALKKTARQLNIVYFLGSDTEPVPDYERRLSELLLYLQQFYGKEMQRHGYGARSFGLDIKSPGRVNIIEYKAKNPAAHYPYENGGGWKAAQELDEFFKAHPDRKKSQHTLIIMPTWNDEKNGPDNPGGVPFYGMGRNCFALDYPAFDIKHLGQKTREGRLLTKWYGGMAHELGHGLNLPHNHQTASDGKKYGTALMGSGNYTFGTSPTFLTPASCALLDACEVFSVTPSQQFYEGKPEVEVGDVAISFKGDQILVSGNYKSPQTVKALNVYIQDPPYAVNQDYDAVSFSRRLGKKSGKFSMKIDKKELEGLNNNEFRISLMFILANGLHMQKHFTFHWDALQDYRDGSKS

SEQ ID NO: 2 - protein, 371 aa, Artificial Sequence
  LS (N terminal methionine and a C-terminal linker + His6 tag)
MEVTVPDALKDRIALKKTARQLNIVYFLGSDTEPVPDYERRLSELLLYLQQFYGKEMQRHGYGARSFGLDIKSPGRVNIIEYKAKNPAAHYPYENGGGWKAAQELDEFFKAHPDRKKSQHTLIIMPTWNDEKNGPDNPGGVPFYGMGRNCFALDYPAFDIKHLGQKTREGRLLTKWYGGMAHELGHGLNLPHNHQTASDGKKYGTALMGSGNYTFGTSPTFLTPASCALLDACEVFSVTPSQQFYEGKPEVEVGDVAISFKGDQILVSGNYKSPQTVKALNVYIQDPPYAVNQDYDAVSFSRRLGKKSGKFSMKIDKKELEGLNNNEFRISLMFILANGLHMQKHFTFHWDALQDYRDGSKSGSGHHHHHH

SEQ ID NO: 3 - DNA, 1116 bp, Artificial Sequence
  Nucleotide sequence of LS
atggaagtcactgtgccggacgccctgaaagatcgcatcgcgctgaagaaaaccgctcgtcagctgaatatcgtctacttcctgggttctgataccgaaccggttccggactacgagcgccgtctgagcgagctgctgttgtatctgcagcaattctatggtaaagaaatgcagcgccatggctatggcgcacgcagctttggtctggacattaagtcaccgggtcgtgtgaacattatcgagtacaaagcgaagaacccggcagcgcattacccgtatgagaatggtggcggctggaaagctgcacaagaactggacgaatttttcaaggcccatccagaccgcaagaaaagccagcacaccctgatcatcatgcctacctggaatgatgagaaaaatggtcctgacaatccgggtggcgttccgttctatggtatgggtcgtaattgttttgcgttggactacccggcgtttgatatcaagcacctgggtcagaaaacgcgtgagggtcgtctgctgacgaaatggtacggtggcatggcgcacgaactgggccacggcctgaatctgccgcacaatcaccagaccgcgagcgatggcaagaaatatggcaccgccctgatgggtagcggcaactacacgttcggtaccagcccgacgttcctgaccccggcgagctgtgcgctgctggatgcctgcgaagtgttcagcgttaccccgagccaacagttttatgagggtaagccagaagtcgaggttggtgatgttgcaatttccttcaagggtgatcaaatcttggtcagcggtaactacaagagcccgcaaaccgtgaaagctctgaacgtttacattcaggatccgccgtacgccgtgaaccaagactacgatgcagtgagctttagccgtcgtctgggcaaaaagtccggtaagtttagcatgaagattgacaaaaaagaactggaaggcctgaataacaacgaattccgtatttccttgatgttcattctggcaaacggcttacacatgcagaagcactttacgtttcactgggatgcgctgcaagactaccgtgacggtagcaaatctggttcgggtcatcatcaccaccatcactga

SEQ ID NO: 4 - protein, 385 aa, Akkermansia muciniphila
MLKRLLSAFFSLFFLGAASGTSFAEVTVPDALKDRIALKKTARQLNIVYFLGSDTEPVPDYERRLSELLLYLQQFYGKEMQRHGYGARSFGLDIKSPGRVNIIEYKAKNPAAHYPYENGGGWKAAQELDEFFKAHPDRKKSQHTLIIMPTWNDEKNGPDNPGGVPFYGMGRNCFALDYPAFDIKHLGQKTREGRLLTKWYGGMAHELGHGLNLPHNHQTASDGKKYGTALMGSGNYTFGTSPTFLTPASCALLDACEVFSVTPSQQFYEGKPEVEVGDVAISFKGDQILVSGNYKSPQTVKALNVYIQDPPYAVNQDYDAVSFSRRLGKKSGKFSMKIDKKELEGLNNNEFRISLMFILANGLHMQKHFTFHWDALQDYRDGSKS

SEQ ID NO: 5 - protein, 361 aa, Artificial Sequence
  Polypeptide capable of binding to O-glycans but lacks or has reduced O-glycoprotein-specific endoprotease activity
EVTVPDALKDRIALKKTARQLNIVYFLGSDTEPVPDYERRLSELLLYLQQFYGKEMQRHGYGARSFGLDIKSPGRVNIIEYKAKNPAAHYPYENGGGWKAAQELDEFFKAHPDRKKSQHTLIIMPTWNDEKNGPDNPGGVPFYGMGRNCFALDYPAFDIKHLGQKTREGRLLTKWYGGMAHALGHGLNLPHNHQTASDGKKYGTALMGSGNYTFGTSPTFLTPASCALLDACEVFSVTPSQQFYEGKPEVEVGDVAISFKGDQILVSGNYKSPQTVKALNVYIQDPPYAVNQDYDAVSFSRRLGKKSGKFSMKIDKKELEGLNNNEFRISLMFILANGLHMQKHFTFHWDALQDYRDGSKS

SEQ ID NO: 6 - protein, 371 aa, Artificial Sequence
  LS E206A (N-terminal methionine and a C-terminal linker + His6 tag)
MEVTVPDALKDRIALKKTARQLNIVYFLGSDTEPVPDYERRLSELLLYLQQFYGKEMQRHGYGARSFGLDIKSPGRVNIIEYKAKNPAAHYPYENGGGWKAAQELDEFFKAHPDRKKSQHTLIIMPTWNDEKNGPDNPGGVPFYGMGRNCFALDYPAFDIKHLGQKTREGRLLTKWYGGMAHALGHGLNLPHNHQTASDGKKYGTALMGSGNYTFGTSPTFLTPASCALLDACEVFSVTPSQQFYEGKPEVEVGDVAISFKGDQILVSGNYKSPQTVKALNVYIQDPPYAVNQDYDAVSFSRRLGKKSGKFSMKIDKKELEGLNNNEFRISLMFILANGLHMQKHFTFHWDALQDYRDGSKSGSGHHHHHH

SEQ ID NO: 7 - DNA, 1116 bp, Artificial Sequence
  Nucleotide sequence encoding LS E206A
atggaagtcactgtgccggacgccctgaaagatcgcatcgcgctgaagaaaaccgctcgtcagctgaatatcgtctacttcctgggttctgataccgaaccggttccggactacgagcgccgtctgagcgagctgctgttgtatctgcagcaattctatggtaaagaaatgcagcgccatggctatggcgcacgcagctttggtctggacattaagtcaccgggtcgtgtgaacattatcgagtacaaagcgaagaacccggcagcgcattacccgtatgagaatggtggcggctggaaagctgcacaagaactggacgaatttttcaaggcccatccagaccgcaagaaaagccagcacaccctgatcatcatgcctacctggaatgatgagaaaaatggtcctgacaatccgggtggcgttccgttctatggtatgggtcgtaattgttttgcgttggactacccggcgtttgatatcaagcacctgggtcagaaaacgcgtgagggtcgtctgctgacgaaatggtacggtggcatggcgcacgcgctgggccacggcctgaatctgccgcacaatcaccagaccgcgagcgatggcaagaaatatggcaccgccctgatgggtagcggcaactacacgttcggtaccagcccgacgttcctgaccccggcgagctgtgcgctgctggatgcctgcgaagtgttcagcgttaccccgagccaacagttttatgagggtaagccagaagtcgaggttggtgatgttgcaatttccttcaagggtgatcaaatcttggtcagcggtaactacaagagcccgcaaaccgtgaaagctctgaacgtttacattcaggatccgccgtacgccgtgaaccaagactacgatgcagtgagctttagccgtcgtctgggcaaaaagtccggtaagtttagcatgaagattgacaaaaaagaactggaaggcctgaataacaacgaattccgtatttccttgatgttcattctggcaaacggcttacacatgcagaagcactttacgtttcactgggatgcgctgcaagactaccgtgacggtagcaaatctggttcgggtcatcatcaccaccatcactga

SEQ ID NO: 8 - protein, 10 aa, Artificial Sequence
  Metalloprotease domain motif
GMAHELGHGL

SEQ ID NO: 9 - protein, 595 aa, Akkermansia muciniphila
MKNLLFALLTGSFCCCYAQQKAAPVPEPEVVATPPADAGRGLIRVDSREIRHYSGTRKEPDYLVSRDNGKTWEMKAAPAGYPPNYGGIPKESPAIVRNPLTREFIRVQPIGGFVFLSRGGLDGKWLAVTNDGKLEEDWKDPEKRKNLKKLGGIMRTPVFVNKGRRVIVPFHNMGGGTKFHISDDGGLTWHVSRNGVTSPRHEARPPHQGVRWFNNAVEATVLEMKDGTLWALARTSQDQAWQAFSKDYGETWSKPEPSRFFGTLTMNTLGRLDDGTIVSLWTNTMALPENATAGNGTWEDVFTNRDSHHIAMSGDEGKTWYGFREIILDEHRNHPGYATLDGPEDRGKHQSEMVQLDKNRILISLGQHKNHRRLVIVDRRWVGAKTRATQTGKDLDSQWTIHTYIPQKKGHCSYNRKPSAELVQDPSGGTKKVLQIKRLDDPELVNEKSNVDYRNGGATWNFPNGTTGLVKFRFRVVDGEQADDSGLQVSLTDRLFNACDSTTKDYALFTFPIRLKPAPHLLLGMKKVPFTPGAWHEISLLWQGGQAVVSLDGKKAGTLKMANKSPNGASYIHFISTGSQPDAGILLDTVNARVK

SEQ ID NO: 10 - protein, 577 aa, Akkermansia muciniphila
QQKAAPVPEPEVVATPPADAGRGLIRVDSREIRHYSGTRKEPDYLVSRDNGKTWEMKAAPAGYPPNYGGIPKESPAIVRNPLTREFIRVQPIGGFVFLSRGGLDGKWLAVTNDGKLEEDWKDPEKRKNLKKLGGIMRTPVFVNKGRRVIVPFHNMGGGTKFHISDDGGLTWHVSRNGVTSPRHEARPPHQGVRWFNNAVEATVLEMKDGTLWALARTSQDQAWQAFSKDYGETWSKPEPSRFFGTLTMNTLGRLDDGTIVSLWTNTMALPENATAGNGTWEDVFTNRDSHHIAMSGDEGKTWYGFREIILDEHRNHPGYATLDGPEDRGKHQSEMVQLDKNRILISLGQHKNHRRLVIVDRRWVGAKTRATQTGKDLDSQWTIHTYIPQKKGHCSYNRKPSAELVQDPSGGTKKVLQIKRLDDPELVNEKSNVDYRNGGATWNFPNGTTGLVKFRFRVVDGEQADDSGLQVSLTDRLFNACDSTTKDYALFTFPIRLKPAPHLLLGMKKVPFTPGAWHEISLLWQGGQAVVSLDGKKAGTLKMANKSPNGASYIHFISTGSQPDAGILLDTVNARVK

SEQ ID NO: 11 - protein, 589 aa, Artificial Sequence
  Am1757 (N-terminal methionine and a C-terminal linker + His6 tag)
MQQKAAPVPEPEVVATPPADAGRGLIRVDSREIRHYSGTRKEPDYLVSRDNGKTWEMKAAPAGYPPNYGGIPKESPAIVRNPLTREFIRVQPIGGFVFLSRGGLDGKWLAVTNDGKLEEDWKDPEKRKNLKKLGGIMRTPVFVNKGRRVIVPFHNMGGGTKFHISDDGGLTWHVSRNGVTSPRHEARPPHQGVRWFNNAVEATVLEMKDGTLWALARTSQDQAWQAFSKDYGETWSKPEPSRFFGTLTMNTLGRLDDGTIVSLWTNTMALPENATAGNGTWEDVFTNRDSHHIAMSGDEGKTWYGFREIILDEHRNHPGYATLDGPEDRGKHQSEMVQLDKNRILISLGQHKNHRRLVIVDRRWVGAKTRATQTGKDLDSQWTIHTYIPQKKGHCSYNRKPSAELVQDPSGGTKKVLQIKRLDDPELVNEKSNVDYRNGGATWNFPNGTTGLVKFRFRVVDGEQADDSGLQVSLTDRLFNACDSTTKDYALFTFPIRLKPAPHLLLGMKKVPFTPGAWHEISLLWQGGQAVVSLDGKKAGTLKMANKSPNGASYIHFISTGSQPDAGILLDTVNARVKGSGLEHHHHHH

SEQ ID NO: 12 - protein, 419 aa, Akkermansia muciniphila
MTWLLCGRGKWNKVKRMMNSVFKCLMSAVCAVALPAFGQEEKTGFPTDRAVTVFSAGEGNPYASIRIPALLSIGKGQLLAFAEGRYKNTDQGENDIIMSVSKNGGKTWSRPRAIAKAHGATFNNPCPVYDAKTRTVTVVFQRYPAGVKERQPNIPDGWDDEKCIRNFMIQSRNGGSSWTKPQEITKTTKRPSGVDIMASGPNAGTQLKSGAHKGRLVIPMNEGPFGKWVISCIYSDDGGKSWKLGQPTANMKGMVNETSIAETDNGGVVMVARHWGAGNCRRIAWSQDGGETWGQVEDAPELFCDSTQNSLMTYSLSDQPAYGGKSRILFSGPSAGRRIKGQVAMSYDNGKTWPVKKLLGEGGFAYSSLAMVEPGIVGVLYEENQEHIKKLKFVPITMEWLTDGEDTGLAPGKKAPVLK

SEQ ID NO: 13 - protein, 381 aa, Akkermansia muciniphila
QEEKTGFPTDRAVTVFSAGEGNPYASIRIPALLSIGKGQLLAFAEGRYKNTDQGENDIIMSVSKNGGKTWSRPRAIAKAHGATFNNPCPVYDAKTRTVTVVFQRYPAGVKERQPNIPDGWDDEKCIRNFMIQSRNGGSSWTKPQEITKTTKRPSGVDIMASGPNAGTQLKSGAHKGRLVIPMNEGPFGKWVISCIYSDDGGKSWKLGQPTANMKGMVNETSIAETDNGGVVMVARHWGAGNCRRIAWSQDGGETWGQVEDAPELFCDSTQNSLMTYSLSDQPAYGGKSRILFSGPSAGRRIKGQVAMSYDNGKTWPVKKLLGEGGFAYSSLAMVEPGIVGVLYEENQEHIKKLKFVPITMEWLTDGEDTGLAPGKKAPVLK

SEQ ID NO: 14 - protein, 393 aa, Artificial Sequence
  Am0707 (including N-terminal methionine and a C-terminal linker + His6 tag)
MQEEKTGFPTDRAVTVFSAGEGNPYASIRIPALLSIGKGQLLAFAEGRYKNTDQGENDIIMSVSKNGGKTWSRPRAIAKAHGATFNNPCPVYDAKTRTVTVVFQRYPAGVKERQPNIPDGWDDEKCIRNFMIQSRNGGSSWTKPQEITKTTKRPSGVDIMASGPNAGTQLKSGAHKGRLVIPMNEGPFGKWVISCIYSDDGGKSWKLGQPTANMKGMVNETSIAETDNGGVVMVARHWGAGNCRRIAWSQDGGETWGQVEDAPELFCDSTQNSLMTYSLSDQPAYGGKSRILFSGPSAGRRIKGQVAMSYDNGKTWPVKKLLGEGGFAYSSLAMVEPGIVGVLYEENQEHIKKLKFVPITMEWLTDGEDTGLAPGKKAPVLKGSGLEHHHHHH

SEQ ID NO: 15 - protein, 2133 aa, Streptococcus oralis
MDKRFFEKRCKFSIRKFTLGVASVMIGATFFAASPVLADQARVGSTDNLPSELADLDKKASDEGHDFDKEAAAQNPGSAETTEGPQTEEELLAQEKEKSEKPSNLPKELEDKLEKAEDNGREVDKDQLAQDTGKLVPEDVAKTTNGELNYGATVKIKTPSGEGSGIVVAKDLVLTVSHNFIKDSQEGNIRKVVDNDQGDGDIYSISYPGLPDVKFSKKDIIHWDREGYLKGFKNDLALVRLRTVLENTPVEVTKKPVVKKIGDKLHVFGYPEGKLNPIVNTTVDFAEPYGEGVQGIGYQGGKPGASGGGIFDTEGKLVGVHQNGVVGKRSGGILFSPAQLKWIQDHMQGISSVKPADLEEKEKPAEEKPKEDKPAAAKPETPKAVTPEWQTVANKEQQGTVTIREEKGVRYNQLSSTAQNDNDGKPALFEKQGLTVDANGNATVDLTFKDDSEKGKSRFGVFLKFKDTKNNVFVGYDQGGWFWEYKTPGNSTWYKGNRVAAPEPGSVNRLSITLKSDGQLNASNNDVNLFDTVTLPGAVNENLKNEKKILLKAGTYSNDRTVVSVKTDNQEGVKADDTPAQKETGPAVDDSKVTYDTIQSKVLKAVIDQAFPRVKEYTLNGHTLPGQVQQFNQVFINNHRITPEVTYKKINETTAEYLMKLRDDAHLINAEMTVRLQVVDNQLHFDVTKIVNHNQVTPGQKIDDERKLLSTISFLGNALVSVSSDQAGAKFDGATMSNNTHVSGDDHIDVTNPMKDLAKGYMYGFVSTDKLAAGVWSNSQNSYGGGSNDWTRLTAYKETVGNANYVGIHSSEWQWEKAYKGIVFPEYTKELPSAKVVITEDANADNKVDWQDGAIAYRSIMNNPQGWEKVKDITAYRIAMNFGSQAQNPFLMTLDGIKKINLHTDGLGQGVLLKGYGSEGHDSGHLNYADIGKRIGGVEDFKTLIEKAKKYGAHLGIHVNASETYPESKYFNENILRKNPDGSYSYGWNWLDQGINIDAAYDLAHGRLARWEDLKKKLGEGLDFIYVDVWGNGQSGDNGAWATHVLAKEINKQGWRFAIEWGHGGEYDSTFQHWAADLTYGGYTNKGINSAITRFIRNHQKDSWVGDYRSYGGAANYPLLGGYSMKDFEGWQGRSDYNGYVTNLFAHDVMTKYFQHFTVSKWENGTPVTMTDNGSTYKWTPEMKVELVDAAGNKVVVTRKSNDVNSPQYRERTVTLNGRVIQDGSAYLTPWNWDANGKKLPTEKEKMYYFNTQAGATTWTLPSDWANSKVYLYKLTDQGKTEEQELTVTDGKITLDLLANQPYVLYRSKQTNPEMSWSEGMHIYDQGFNSGTLKHWTISGDASKAEIVKSQGANEMLRIQGNKSKVSLTQKLTGLKPNTKYAVYVGVDNRSNAKASITVNTGEKEVTTYTNKSLALNYIKAYAHNNRRENATVDDTSYFQNMYAFFTTGSDVSNVTLTLSREAGDEATYFDEIRTFENNSSMYGDKHDTGQGTFKQDFENVAQGIFPFVVGGVEGVEDNRTHLSEKHDPYTQRGWNGKKVDDVIEGNWSLKTNGLVSRRNLVYQTIPQNFRFEAGKTYRVTFEYEAGSDNTYAFVVGKGEFQSGRRGTQASNLEMHELPNTWTDSKKAKKVTFLVTGAETGDTWVGIYSTGNASNTRGDAGGNANFRGYNDFMMDNLQIEEITLTGKMLTENALKNYLPTVAMTNYTKESMDALKEAVFNLSQADDDISVEEARAEIAKIEALKNALVQKKTALVAEDFESLDAPAQPGEGLENAFDGNVSSLWHTSWNGGDVGKPATMVLKEPTEITGLRYVPRASDSNGNLRDVKLVVTDESGKEHTFNVTDWPNNNKPKDIDFGKTIKAKKIVLTGTKTYGDGGDKYQSAAELIFTRPQVAETPLDLSGYEAALAKAQKLTDKDNQEEVASVQASMKYATDNHLLTERMVAYFADYLNQLKDSATKPDAPTSSKGEEQPPVLDVPEFKGGVNATEAAVHEVPEFKGGVNAVQALVHELPEYKGGANAVLAAANEVPEYKGGANAVEALVNEKPAYTGVLATAGDQAAPTVEKPEYPLTPSPVADTKTPGAKDEEKLPATGEHSSEVALFLASVSIALSAAVLATKRKEEGSGLEHHHHHH

SEQ ID NO: 16 - DNA, 22 bp, Artificial Sequence
  E206A forward primer
atggcgcacgcgctgggccacg

SEQ ID NO: 17 - DNA, 19 bp, Artificial Sequence
  E206A reverse primer
gccaccgtaccatttcgtc

SEQ ID NO: 18 - protein, 166 aa, Artificial Sequence
  EPO
APPRLICDSRVLERYLLEAKEAEDITTGCAEHCSLDENITVPDTKVDFYAWKRMEVGQQAVEVWQGLALLSEAVLRGQALLVNSSQPWEPLQLHVDKAVSGLRSLTTLLRALGAQKEAISPPDAASAAPLRTITADTFRKLFRVYSNFLRGKLKLYTGEACRTGDR

SEQ ID NO: 19 - skipped

SEQ ID NO: 20 - protein, 361 aa, Artificial Sequence
  Polypeptide capable of binding to O-glycans but lacks or has reduced O-glycoprotein-specific endoprotease activity
EVTVPDALKDRIALKKTARQLNIVYFLGSDTEPVPDYERRLSELLLYLQQFYGKEMQRHGYGARSFGLDIKSPGRVNIIEYKAKNPAAHYPYENGGGWKAAQELDEFFKAHPDRKKSQHTLIIMPTWNDEKNGPDNPGGVPFYGMGRNCFALDYPAFDIKHLGQKTREGRLLTKWYGGMAAALGHGLNLPHNHQTASDGKKYGTALMGSGNYTFGTSPTFLTPASCALLDACEVFSVTPSQQFYEGKPEVEVGDVAISFKGDQILVSGNYKSPQTVKALNVYIQDPPYAVNQDYDAVSFSRRLGKKSGKFSMKIDKKELEGLNNNEFRISLMFILANGLHMQKHFTFHWDALQDYRDGSKS

SEQ ID NO: 21 - protein, 371 aa, Artificial Sequence
  LS HE206AA or LS H205A/E206A (including N-terminal methionine and C-terminal linker)
MEVTVPDALKDRIALKKTARQLNIVYFLGSDTEPVPDYERRLSELLLYLQQFYGKEMQRHGYGARSFGLDIKSPGRVNIIEYKAKNPAAHYPYENGGGWKAAQELDEFFKAHPDRKKSQHTLIIMPTWNDEKNGPDNPGGVPFYGMGRNCFALDYPAFDIKHLGQKTREGRLLTKWYGGMAAALGHGLNLPHNHQTASDGKKYGTALMGSGNYTFGTSPTFLTPASCALLDACEVFSVTPSQQFYEGKPEVEVGDVAISFKGDQILVSGNYKSPQTVKALNVYIQDPPYAVNQDYDAVSFSRRLGKKSGKFSMKIDKKELEGLNNNEFRISLMFILANGLHMQKHFTFHWDALQDYRDGSKSGSGHHHHHH

SEQ ID NO: 22 - DNA, 1116 bp, Artificial Sequence
  Nucleotide sequence encoding LS HE206AA or LS H205A/E206A
atggaagtcactgtgccggacgccctgaaagatcgcatcgcgctgaagaaaaccgctcgtcagctgaatatcgtctacttcctgggttctgataccgaaccggttccggactacgagcgccgtctgagcgagctgctgttgtatctgcagcaattctatggtaaagaaatgcagcgccatggctatggcgcacgcagctttggtctggacattaagtcaccgggtcgtgtgaacattatcgagtacaaagcgaagaacccggcagcgcattacccgtatgagaatggtggcggctggaaagctgcacaagaactggacgaatttttcaaggcccatccagaccgcaagaaaagccagcacaccctgatcatcatgcctacctggaatgatgagaaaaatggtcctgacaatccgggtggcgttccgttctatggtatgggtcgtaattgttttgcgttggactacccggcgtttgatatcaagcacctgggtcagaaaacgcgtgagggtcgtctgctgacgaaatggtacggtggcatggcggccgcgctgggccacggcctgaatctgccgcacaatcaccagaccgcgagcgatggcaagaaatatggcaccgccctgatgggtagcggcaactacacgttcggtaccagcccgacgttcctgaccccggcgagctgtgcgctgctggatgcctgcgaagtgttcagcgttaccccgagccaacagttttatgagggtaagccagaagtcgaggttggtgatgttgcaatttccttcaagggtgatcaaatcttggtcagcggtaactacaagagcccgcaaaccgtgaaagctctgaacgtttacattcaggatccgccgtacgccgtgaaccaagactacgatgcagtgagctttagccgtcgtctgggcaaaaagtccggtaagtttagcatgaagattgacaaaaaagaactggaaggcctgaataacaacgaattccgtatttccttgatgttcattctggcaaacggcttacacatgcagaagcactttacgtttcactgggatgcgctgcaagactaccgtgacggtagcaaatctggttcgggtcatcatcaccaccatcactga

SEQ ID NO: 23 - protein, 10 aa, Artificial Sequence
  disrupted metalloprotease motif
GMAHALGHGL

SEQ ID NO: 24 - protein, 10 aa, Artificial Sequence
  disrupted metalloprotease motif
GMAAELGHGL

SEQ ID NO: 25 - protein, 10 aa, Artificial Sequence
  disrupted metalloprotease motif
GMAAALGHGL

SEQ ID NO: 26 - protein, 882 aa, Pseudomonas aeruginosa
ATQEEILDAALVSGDSSQLTDSHLVALRLQQQVERIRQTRTQLLDGLYQNLSQAYDPGAASMWVLPANPDNTLPFLIGDKGRVLASLSLEAGGRGLAYGTNVLTQLSGTNAAHAPLLKRAVQWLVNGDPGAATAKDFKVSVVGVDKTAALNGLKSAGLQPADAACNALTDASCASTSKLLVLGNGASAASLSATVRARLQAGLPILFVHTNGWNQSSTGQQILAGLGLQEGPYGGNYWDKDRVPSSRTRTRSVELGGAYGQDPALVQQIVDGSWRTDYDWSKCTSYVGRTTCDDVPGLSDFSKRVDVLKGALDAYNQKAQNLFALPGTTSLRLWLLWADAVRQNIRYPMDKAADTARFQETFVADAIVGYVREAGAAQKELGSYAGQRQQSMPVSGSEETLTLTLPSAQGFTAIGRMAAPGKRLSIRIEDAGQASLAVGLNTQRIGSTRLWNTRQYDRPRFLKSPDIKLQANQSVALVSPYGGLLQLVYSGATPGQTVTVKVTGAASQPFLDIQPGEDSSQAIADFIQALDADKADWLEIRSGSVEVHAKVEKVRGSIDKDYGGDVQRFIRELNEVFIDDAYTLAGFAIPNQAKTPAIQQECAARGWDCDSETLHKLPGTQHINVDQYAQCGGGCSGNPYDQTWGLNPRGWGESHELGHNLQVNRLKVYGGRSGEISNQIFPLHKDWRVLREFGQNLDDTRVNYRNAYNLIVAGRAEADPLAGVYKRLWEDPGTYALNGERMAFYTQWVHYWADLKNDPLQGWDIWTLLYLHQRQVDKSDWDANKAALGYGTYAQRPGNSGDASSTDGNDNLLLGLSWLTQRDQRPTFALWGIRTSAAAQAQVAAYGFAEQPAFFYANNRTNEYSTVKLLDMSQGSPAWPFP

SEQ ID NO: 27 - protein, 536 aa, Bacteroides thetaiotaomicron
DKWEKEFRIRSYEPYSNIAEWADKLMTKKYSDLDNPTGISVKAGDDIIVLVGDTYGQNISMQCIWETGTEYKQTASSGDVYMLNPGVNKLTMKGEGQLFVMYNTELTSNTAKPIKIHIPLGSGTVNGFFDLKEHKTDEKYAELLKKSTHKYFCIRGEKIMFYFHRNKLLEYVPNNILSAIHLWDNIVGWQQELMGIDDVRPSQVNNHLFAISPEGSYMWASDYQIGFVYTYLGNILLEDNVMAAEDNAWGPAHEIGHVHQAAINWASSTESSNNLFSNFIIYKLGKYKSRGNGLGSVATARYANGQAWYNMGDATHQNEDTETHMRMNWQLWIYYHRCEYKTDFWQTLFKLMREVNMTEGEDPGKKQLEFAKMASKAANQNLTDFFEMWGFFEPVNTTIEQYGTYKYYVSDAMIREAKEYMAQFPAPKHAFQYIEDRKKSEFPSNDYRYSAVGDVGYYTQFKENQKITKAITAELAGRKVSIQNGDEAVAFELRENDENGKLLYFSTFTTFEIPSSILMVNAKLYAVQADGKRILL

SEQ ID NO: 28 - protein, 507 aa, Clostridium perfringens
VLELEMRGDSISEAKKRKVWNFQDWQITGLSARAGDKITVYVDVAEGDPTPTLLYKQSLTQHGGATSFQLKPGKNEITIPEINYESNGIPKDVIQGGDLFFTNYKSDSQKRAPKVRIEGASKYPVFILGKSDENEVMKELEAYVEKIKAEPKTTPNIFAVSSNKSLEFVQATYALDWYKKNNKTPKYTAEQWDQYIADAMGFWGFDNSKDVNSDFNFRIMPMVKNLSGGAFMNAGNGVIGIRPGNQDAILAANKGWGVAHELGHNFDTGGRTIVEVTNNMMPLFFESKYKTKTRITDQNIWENNTYPKVGLDDYSNNELYNKADSTHLAQLAPLWQLYLYDNTFYGKFERQFRERDFGNKNREDIYKSWVVAASDAMELDLTEFFARHGIRVDDKVKEDLAKYPKPDKKIYYLNDLAMNYKGDGFTENAKVSVSTSGSNGNIKLSFSVDDENKDNILGYEIRRDGKYVGFTSNDSFVDTKSNLDEDGVYVVTPYDRKLNTLNPIEVN

SEQ ID NO: 29 - protein, 892 aa, Artificial Sequence
  polypeptide having O-glycoprotein-specific endoprotease activity (including N-terminal methionine and a C-terminal linker + His6 tag)
MATQEEILDAALVSGDSSQLTDSHLVALRLQQQVERIRQTRTQLLDGLYQNLSQAYDPGAASMWVLPANPDNTLPFLIGDKGRVLASLSLEAGGRGLAYGTNVLTQLSGTNAAHAPLLKRAVQWLVNGDPGAATAKDFKVSVVGVDKTAALNGLKSAGLQPADAACNALTDASCASTSKLLVLGNGASAASLSATVRARLQAGLPILFVHTNGWNQSSTGQQILAGLGLQEGPYGGNYWDKDRVPSSRTRTRSVELGGAYGQDPALVQQIVDGSWRTDYDWSKCTSYVGRTTCDDVPGLSDFSKRVDVLKGALDAYNQKAQNLFALPGTTSLRLWLLWADAVRQNIRYPMDKAADTARFQETFVADAIVGYVREAGAAQKELGSYAGQRQQSMPVSGSEETLTLTLPSAQGFTAIGRMAAPGKRLSIRIEDAGQASLAVGLNTQRIGSTRLWNTRQYDRPRFLKSPDIKLQANQSVALVSPYGGLLQLVYSGATPGQTVTVKVTGAASQPFLDIQPGEDSSQAIADFIQALDADKADWLEIRSGSVEVHAKVEKVRGSIDKDYGGDVQRFIRELNEVFIDDAYTLAGFAIPNQAKTPAIQQECAARGWDCDSETLHKLPGTQHINVDQYAQCGGGCSGNPYDQTWGLNPRGWGESHELGHNLQVNRLKVYGGRSGEISNQIFPLHKDWRVLREFGQNLDDTRVNYRNAYNLIVAGRAEADPLAGVYKRLWEDPGTYALNGERMAFYTQWVHYWADLKNDPLQGWDIWTLLYLHQRQVDKSDWDANKAALGYGTYAQRPGNSGDASSTDGNDNLLLGLSWLTQRDQRPTFALWGIRTSAAAQAQVAAYGFAEQPAFFYANNRTNEYSTVKLLDMSQGSPAWPFPGSGHHHHHH

SEQ ID NO: 30 - protein, 546 aa, Artificial Sequence
  polypeptide having O-glycoprotein-specific endoprotease activity (including N-terminal methionine and a C-terminal linker + His6 tag)
MDKWEKEFRIRSYEPYSNIAEWADKLMTKKYSDLDNPTGISVKAGDDIIVLVGDTYGQNISMQCIWETGTEYKQTASSGDVYMLNPGVNKLTMKGEGQLFVMYNTELTSNTAKPIKIHIPLGSGTVNGFFDLKEHKTDEKYAELLKKSTHKYFCIRGEKIMFYFHRNKLLEYVPNNILSAIHLWDNIVGWQQELMGIDDVRPSQVNNHLFAISPEGSYMWASDYQIGFVYTYLGNILLEDNVMAAEDNAWGPAHEIGHVHQAAINWASSTESSNNLFSNFIIYKLGKYKSRGNGLGSVATARYANGQAWYNMGDATHQNEDTETHMRMNWQLWIYYHRCEYKTDFWQTLFKLMREVNMTEGEDPGKKQLEFAKMASKAANQNLTDFFEMWGFFEPVNTTIEQYGTYKYYVSDAMIREAKEYMAQFPAPKHAFQYIEDRKKSEFPSNDYRYSAVGDVGYYTQFKENQKITKAITAELAGRKVSIQNGDEAVAFELRENDENGKLLYFSTFTTFEIPSSILMVNAKLYAVQADGKRILLGSGHHHHHH

SEQ ID NO: 31 - protein, 517 aa, Artificial Sequence
  polypeptide having O-glycoprotein-specific endoprotease activity (including N-terminal methionine and a C-terminal linker + His6 tag)
MVLELEMRGDSISEAKKRKVWNFQDWQITGLSARAGDKITVYVDVAEGDPTPTLLYKQSLTQHGGATSFQLKPGKNEITIPEINYESNGIPKDVIQGGDLFFTNYKSDSQKRAPKVRIEGASKYPVFILGKSDENEVMKELEAYVEKIKAEPKTTPNIFAVSSNKSLEFVQATYALDWYKKNNKTPKYTAEQWDQYIADAMGFWGFDNSKDVNSDFNFRIMPMVKNLSGGAFMNAGNGVIGIRPGNQDAILAANKGWGVAHELGHNFDTGGRTIVEVTNNMMPLFFESKYKTKTRITDQNIWENNTYPKVGLDDYSNNELYNKADSTHLAQLAPLWQLYLYDNTFYGKFERQFRERDFGNKNREDIYKSWVVAASDAMELDLTEFFARHGIRVDDKVKEDLAKYPKPDKKIYYLNDLAMNYKGDGFTENAKVSVSTSGSNGNIKLSFSVDDENKDNILGYEIRRDGKYVGFTSNDSFVDTKSNLDEDGVYVVTPYDRKLNTLNPIEVNGSGHHHHHH

SEQ ID NO: 32 - protein, 923 aa, Pseudomonas aeruginosa
MSLSTTAFPSLQGENMSRSPIPRHRALLAGFCLAGALSAQAATQEEILDAALVSGDSSQLTDSHLVALRLQQQVERIRQTRTQLLDGLYQNLSQAYDPGAASMWVLPANPDNTLPFLIGDKGRVLASLSLEAGGRGLAYGTNVLTQLSGTNAAHAPLLKRAVQWLVNGDPGAATAKDFKVSVVGVDKTAALNGLKSAGLQPADAACNALTDASCASTSKLLVLGNGASAASLSATVRARLQAGLPILFVHTNGWNQSSTGQQILAGLGLQEGPYGGNYWDKDRVPSSRTRTRSVELGGAYGQDPALVQQIVDGSWRTDYDWSKCTSYVGRTTCDDVPGLSDFSKRVDVLKGALDAYNQKAQNLFALPGTTSLRLWLLWADAVRQNIRYPMDKAADTARFQETFVADAIVGYVREAGAAQKELGSYAGQRQQSMPVSGSEETLTLTLPSAQGFTAIGRMAAPGKRLSIRIEDAGQASLAVGLNTQRIGSTRLWNTRQYDRPRFLKSPDIKLQANQSVALVSPYGGLLQLVYSGATPGQTVTVKVTGAASQPFLDIQPGEDSSQAIADFIQALDADKADWLEIRSGSVEVHAKVEKVRGSIDKDYGGDVQRFIRELNEVFIDDAYTLAGFAIPNQAKTPAIQQECAARGWDCDSETLHKLPGTQHINVDQYAQCGGGCSGNPYDQTWGLNPRGWGESHELGHNLQVNRLKVYGGRSGEISNQIFPLHKDWRVLREFGQNLDDTRVNYRNAYNLIVAGRAEADPLAGVYKRLWEDPGTYALNGERMAFYTQWVHYWADLKNDPLQGWDIWTLLYLHQRQVDKSDWDANKAALGYGTYAQRPGNSGDASSTDGNDNLLLGLSWLTQRDQRPTFALWGIRTSAAAQAQVAAYGFAEQPAFFYANNRTNEYSTVKLLDMSQGSPAWPFP

SEQ ID NO: 33 - protein, 857 aa, Bacteroides thetaiotaomicron
MTIKRFITNLLALFTLFTVSLACKDTEKSIINSSFSISEEYLIQNLDKSSTSVQIPINTSMELAQWSVSYEANWLQCSKQKTAAEGTFLRITVNENTGETKRTANIKVTSTTATYTITVNQYAKGEVIVEGDIKVTPTGGKASEHQEGQDIENTYDGKFSTDGAAPFHTPWGQSAKFPVTLEYYFKGDTEIDYLIYYTRSGNGNFGKVKVYTTTNPDRSDYTLQGEYDFKEQNAPSKVSFSEGIKATGIKFEVLSGLGDFVSCDEMEFYKTNTDKTLDKQLLTVFTDITCTEIKNNVTNEQIQALPDYFVRIAEAVRDNTYDKWEKEFRIRSYEPYSNIAEWADKLMTKKYSDLDNPTGISVKAGDDIIVLVGDTYGQNISMQCIWETGTEYKQTASSGDVYMLNPGVNKLTMKGEGQLFVMYNTELTSNTAKPIKIHIPLGSGTVNGFFDLKEHKTDEKYAELLKKSTHKYFCIRGEKIMFYFHRNKLLEYVPNNILSAIHLWDNIVGWQQELMGIDDVRPSQVNNHLFAISPEGSYMWASDYQIGFVYTYLGNILLEDNVMAAEDNAWGPAHEIGHVHQAAINWASSTESSNNLFSNFIIYKLGKYKSRGNGLGSVATARYANGQAWYNMGDATHQNEDTETHMRMNWQLWIYYHRCEYKTDFWQTLFKLMREVNMTEGEDPGKKQLEFAKMASKAANQNLTDFFEMWGFFEPVNTTIEQYGTYKYYVSDAMIREAKEYMAQFPAPKHAFQYIEDRKKSEFPSNDYRYSAVGDVGYYTQFKENQKITKAITAELAGRKVSIQNGDEAVAFELRENDENGKLLYFSTFTTFEIPSSILMVNAKLYAVQADGKRILL

SEQ ID NO: 34 - protein, 1687 aa, Clostridium perfringens
MNKRKIAAIILATMITNLSATTIDVLAQELNTKNNSKVEVSHDDESHQARVSKFDLYNSDKLDAYNQEFQVSRSNIKSINNNGGKYNSSTIDKAIDGNLETHWETGKPNDANFTNEVVVTFNEITNIDRIVYSARRDSARGKGFAKEFEIYASLKDEGDDFNLVSSGEYTESTRDLVEIKFNPTDFKRLKFKFKKADQNWASAAEFMFYKEDKLNEKFNGLFTDSSMNKVSEEFNTLEKLNAFENELKDHPIYDLYKEGLNNARAILTETSENPTKATLGQITYNLNDDYNNQYRMPYKNIKAIKNNGRHYAAQNIEKAIDNDVNTYWETGTLNSSSFNNEVEVEFNDLVTLDRIVYGSRQSDLKGFAEEVYIYASRTSKGDTYKLVATGAHEATKGLVEAKFEPTEFKRVKFKFKKSKQNSATLNELMFYKPDEVYSSIPKLFTDGTMSELSEEFNSLEKINAFKEKAKNHPLYNDFNETIELAESLISNPRKEDVLELEMRGDSISEAKKRKVWNFQDWQITGLSARAGDKITVYVDVAEGDPTPTLLYKQSLTQHGGATSFQLKPGKNEITIPEINYESNGIPKDVIQGGDLFFTNYKSDSQKRAPKVRIEGASKYPVFILGKSDENEVMKELEAYVEKIKAEPKTTPNIFAVSSNKSLEFVQATYALDWYKKNNKTPKYTAEQWDQYIADAMGFWGFDNSKDVNSDFNFRIMPMVKNLSGGAFMNAGNGVIGIRPGNQDAILAANKGWGVAHELGHNFDTGGRTIVEVTNNMMPLFFESKYKTKTRITDQNIWENNTYPKVGLDDYSNNELYNKADSTHLAQLAPLWQLYLYDNTFYGKFERQFRERDFGNKNREDIYKSWVVAASDAMELDLTEFFARHGIRVDDKVKEDLAKYPKPDKKIYYLNDLAMNYKGDGFTENAKVSVSTSGSNGNIKLSFSVDDENKDNILGYEIRRDGKYVGFTSNDSFVDTKSNLDEDGVYVVTPYDRKLNTLNPIEVNALQPTLSVNPVITLALGEEFNEEEYIVAKDIKGNSLSESVKVKSSNVNTSKVGEYEVLYSLEDSKGNEYTKTSKVNVVSRKEYMSDLTPKQSSNGWGTVRKDKSISGGVIGLTRDGDFVDYNKGLGLHSNAEYVYDLEGKDYDYFESYVGVDKAMSSRPASSVIFKVLVDGEEKFNSGVMRSTTPQKYVKVDVKNAKELKLIVNDAGDGDSSDHASFGDAKLATLSSKPIIKGENLAYSMDEKVDLMKGITATDIEDGNITSKVQIKSSDFVEGKSGIFTVVYSVTDSDGLTSECSRTIAVTDKETQLSDLNWKSATIGSGSVRKDRAVSGNQIRLLNEDNSVETFAKGIGTHSYSEIVYNSEGYDIFDTWVGIDRHVADKKVSSVKFKVYVDGELKAETDVMRIDTPKKRLVVDVRNSKEIKLVVDVADNGNNWDHADWADAKFRNLAEYDASELNKAIEEAKKLDLNNYTEESSEALKNAISKGEEALLSKDKETINSALEELNKEMNSLVKVDLNAVINIPDKYLLKSIQNQLNKTGDITLGDMYSLTTLTLSGVEDLTGLENAKNLETLNMDYNEVKDLRPLSKLKKLNTLNAQEQFIAAGELKPSNGKVIGDSKVYNREGKNVAKTIRVVDKNGNTILEQDAKDEFTINTKDLSSGLYGVHVLFEDEGFSGVMFYLFNV

SEQ ID NO: 35 - protein, 882 aa, Artificial Sequence
  Polypeptide capable of binding to O-glycans but lack or has reduced O-glycoprotein-specific endoprotease activity - Pseudomonas aeruginosa PAO1 (double mutant with removed signal sequence)
ATQEEILDAALVSGDSSQLTDSHLVALRLQQQVERIRQTRTQLLDGLYQNLSQAYDPGAASMWVLPANPDNTLPFLIGDKGRVLASLSLEAGGRGLAYGTNVLTQLSGTNAAHAPLLKRAVQWLVNGDPGAATAKDFKVSVVGVDKTAALNGLKSAGLQPADAACNALTDASCASTSKLLVLGNGASAASLSATVRARLQAGLPILFVHTNGWNQSSTGQQILAGLGLQEGPYGGNYWDKDRVPSSRTRTRSVELGGAYGQDPALVQQIVDGSWRTDYDWSKCTSYVGRTTCDDVPGLSDFSKRVDVLKGALDAYNQKAQNLFALPGTTSLRLWLLWADAVRQNIRYPMDKAADTARFQETFVADAIVGYVREAGAAQKELGSYAGQRQQSMPVSGSEETLTLTLPSAQGFTAIGRMAAPGKRLSIRIEDAGQASLAVGLNTQRIGSTRLWNTRQYDRPRFLKSPDIKLQANQSVALVSPYGGLLQLVYSGATPGQTVTVKVTGAASQPFLDIQPGEDSSQAIADFIQALDADKADWLEIRSGSVEVHAKVEKVRGSIDKDYGGDVQRFIRELNEVFIDDAYTLAGFAIPNQAKTPAIQQECAARGWDCDSETLHKLPGTQHINVDQYAQCGGGCSGNPYDQTWGLNPRGWGESAALGHNLQVNRLKVYGGRSGEISNQIFPLHKDWRVLREFGQNLDDTRVNYRNAYNLIVAGRAEADPLAGVYKRLWEDPGTYALNGERMAFYTQWVHYWADLKNDPLQGWDIWTLLYLHQRQVDKSDWDANKAALGYGTYAQRPGNSGDASSTDGNDNLLLGLSWLTQRDQRPTFALWGIRTSAAAQAQVAAYGFAEQPAFFYANNRTNEYSTVKLLDMSQGSPAWPFP

SEQ ID NO: 36 - protein, 536 aa, Artificial Sequence
  Polypeptide capable of binding to O-glycans but lack or has reduced O-glycoprotein-specific endoprotease activity - Bacteroides thetaiotaomicron VPI-5482 (double mutant with removed signal and other immature sequences)
DKWEKEFRIRSYEPYSNIAEWADKLMTKKYSDLDNPTGISVKAGDDIIVLVGDTYGQNISMQCIWETGTEYKQTASSGDVYMLNPGVNKLTMKGEGQLFVMYNTELTSNTAKPIKIHIPLGSGTVNGFFDLKEHKTDEKYAELLKKSTHKYFCIRGEKIMFYFHRNKLLEYVPNNILSAIHLWDNIVGWQQELMGIDDVRPSQVNNHLFAISPEGSYMWASDYQIGFVYTYLGNILLEDNVMAAEDNAWGPAAAIGHVHQAAINWASSTESSNNLFSNFIIYKLGKYKSRGNGLGSVATARYANGQAWYNMGDATHQNEDTETHMRMNWQLWIYYHRCEYKTDFWQTLFKLMREVNMTEGEDPGKKQLEFAKMASKAANQNLTDFFEMWGFFEPVNTTIEQYGTYKYYVSDAMIREAKEYMAQFPAPKHAFQYIEDRKKSEFPSNDYRYSAVGDVGYYTQFKENQKITKAITAELAGRKVSIQNGDEAVAFELRENDENGKLLYFSTFTTFEIPSSILMVNAKLYAVQADGKRILL

SEQ ID NO: 37 - protein, 507 aa, Artificial Sequence
  Polypeptide capable of binding to O-glycans but lack or has reduced O-glycoprotein-specific endoprotease activity - Clostridium perfringens (double mutant with removed signal and other immature sequences)
VLELEMRGDSISEAKKRKVWNFQDWQITGLSARAGDKITVYVDVAEGDPTPTLLYKQSLTQHGGATSFQLKPGKNEITIPEINYESNGIPKDVIQGGDLFFTNYKSDSQKRAPKVRIEGASKYPVFILGKSDENEVMKELEAYVEKIKAEPKTTPNIFAVSSNKSLEFVQATYALDWYKKNNKTPKYTAEQWDQYIADAMGFWGFDNSKDVNSDFNFRIMPMVKNLSGGAFMNAGNGVIGIRPGNQDAILAANKGWGVAAALGHNFDTGGRTIVEVTNNMMPLFFESKYKTKTRITDQNIWENNTYPKVGLDDYSNNELYNKADSTHLAQLAPLWQLYLYDNTFYGKFERQFRERDFGNKNREDIYKSWVVAASDAMELDLTEFFARHGIRVDDKVKEDLAKYPKPDKKIYYLNDLAMNYKGDGFTENAKVSVSTSGSNGNIKLSFSVDDENKDNILGYEIRRDGKYVGFTSNDSFVDTKSNLDEDGVYVVTPYDRKLNTLNPIEVN

SEQ ID NO: 38 - protein, 892 aa, Artificial Sequence
  Polypeptide capable of binding to O-glycans but lack or has reduced O-glycoprotein-specific endoprotease activity - Pseudomonas aeruginosa PAO1 (double mutant with removed signal sequence, with N-term Met, C-term linker/tag)
MATQEEILDAALVSGDSSQLTDSHLVALRLQQQVERIRQTRTQLLDGLYQNLSQAYDPGAASMWVLPANPDNTLPFLIGDKGRVLASLSLEAGGRGLAYGTNVLTQLSGTNAAHAPLLKRAVQWLVNGDPGAATAKDFKVSVVGVDKTAALNGLKSAGLQPADAACNALTDASCASTSKLLVLGNGASAASLSATVRARLQAGLPILFVHTNGWNQSSTGQQILAGLGLQEGPYGGNYWDKDRVPSSRTRTRSVELGGAYGQDPALVQQIVDGSWRTDYDWSKCTSYVGRTTCDDVPGLSDFSKRVDVLKGALDAYNQKAQNLFALPGTTSLRLWLLWADAVRQNIRYPMDKAADTARFQETFVADAIVGYVREAGAAQKELGSYAGQRQQSMPVSGSEETLTLTLPSAQGFTAIGRMAAPGKRLSIRIEDAGQASLAVGLNTQRIGSTRLWNTRQYDRPRFLKSPDIKLQANQSVALVSPYGGLLQLVYSGATPGQTVTVKVTGAASQPFLDIQPGEDSSQAIADFIQALDADKADWLEIRSGSVEVHAKVEKVRGSIDKDYGGDVQRFIRELNEVFIDDAYTLAGFAIPNQAKTPAIQQECAARGWDCDSETLHKLPGTQHINVDQYAQCGGGCSGNPYDQTWGLNPRGWGESAALGHNLQVNRLKVYGGRSGEISNQIFPLHKDWRVLREFGQNLDDTRVNYRNAYNLIVAGRAEADPLAGVYKRLWEDPGTYALNGERMAFYTQWVHYWADLKNDPLQGWDIWTLLYLHQRQVDKSDWDANKAALGYGTYAQRPGNSGDASSTDGNDNLLLGLSWLTQRDQRPTFALWGIRTSAAAQAQVAAYGFAEQPAFFYANNRTNEYSTVKLLDMSQGSPAWPFPGSGHHHHHH

SEQ ID NO: 39 - protein, 546 aa, Artificial Sequence
  Polypeptide capable of binding to O-glycans but lack or has reduced O-glycoprotein-specific endoprotease activity - Bacteroides thetaiotaomicron VPI-5482 (double mutant with removed signal and other sequences from immature protein, with N-term
MDKWEKEFRIRSYEPYSNIAEWADKLMTKKYSDLDNPTGISVKAGDDIIVLVGDTYGQNISMQCIWETGTEYKQTASSGDVYMLNPGVNKLTMKGEGQLFVMYNTELTSNTAKPIKIHIPLGSGTVNGFFDLKEHKTDEKYAELLKKSTHKYFCIRGEKIMFYFHRNKLLEYVPNNILSAIHLWDNIVGWQQELMGIDDVRPSQVNNHLFAISPEGSYMWASDYQIGFVYTYLGNILLEDNVMAAEDNAWGPAAAIGHVHQAAINWASSTESSNNLFSNFIIYKLGKYKSRGNGLGSVATARYANGQAWYNMGDATHQNEDTETHMRMNWQLWIYYHRCEYKTDFWQTLFKLMREVNMTEGEDPGKKQLEFAKMASKAANQNLTDFFEMWGFFEPVNTTIEQYGTYKYYVSDAMIREAKEYMAQFPAPKHAFQYIEDRKKSEFPSNDYRYSAVGDVGYYTQFKENQKITKAITAELAGRKVSIQNGDEAVAFELRENDENGKLLYFSTFTTFEIPSSILMVNAKLYAVQADGKRILLGSGHHHHHH

SEQ ID NO: 40 - protein, 517 aa, Artificial Sequence
  Polypeptide capable of binding to O-glycans but lack or has reduced O-glycoprotein-specific endoprotease activity - Clostridium perfringens (double mutant with removed signal and other sequences from immature protein, with N-term Met, C-term
MVLELEMRGDSISEAKKRKVWNFQDWQITGLSARAGDKITVYVDVAEGDPTPTLLYKQSLTQHGGATSFQLKPGKNEITIPEINYESNGIPKDVIQGGDLFFTNYKSDSQKRAPKVRIEGASKYPVFILGKSDENEVMKELEAYVEKIKAEPKTTPNIFAVSSNKSLEFVQATYALDWYKKNNKTPKYTAEQWDQYIADAMGFWGFDNSKDVNSDFNFRIMPMVKNLSGGAFMNAGNGVIGIRPGNQDAILAANKGWGVAAALGHNFDTGGRTIVEVTNNMMPLFFESKYKTKTRITDQNIWENNTYPKVGLDDYSNNELYNKADSTHLAQLAPLWQLYLYDNTFYGKFERQFRERDFGNKNREDIYKSWVVAASDAMELDLTEFFARHGIRVDDKVKEDLAKYPKPDKKIYYLNDLAMNYKGDGFTENAKVSVSTSGSNGNIKLSFSVDDENKDNILGYEIRRDGKYVGFTSNDSFVDTKSNLDEDGVYVVTPYDRKLNTLNPIEVNGSGHHHHHH

SEQ ID NO: 41 - protein, 5 aa, Artificial Sequence
  Metalloprotease motif
HELGH

SEQ ID NO: 42 - protein, 5 aa, Artificial Sequence
  Metalloprotease motif
HEIGH

SEQ ID NO: 43 - protein, 10 aa, Artificial Sequence
  Metalloprotease motif
GVAHELGHNF

SEQ ID NO: 44 - protein, 5 aa, Artificial Sequence
  disrupted metalloprotease motif
HALGH

SEQ ID NO: 45 - protein, 5 aa, Artificial Sequence
  disrupted metalloprotease motif
AELGH

SEQ ID NO: 46 - protein, 5 aa, Artificial Sequence
  disrupted metalloprotease motif
AALGH

SEQ ID NO: 47 - protein, 19 aa, Artificial Sequence
  glycodrosocin peptide with O-gly site on the T
GKPRPYSPRPTSHPRPIRV

SEQ ID NO: 48 - protein, 7 aa, Artificial Sequence
  Non-O-glycosylated peptide
YIYGSFK

SEQ ID NO: 49 - protein, 7 aa, Artificial Sequence
  Non-O-glycosylated peptide
KKLVFFA

SEQ ID NO: 50 - protein, 14 aa, Artificial Sequence
  Non-O-glycosylated peptide
FLPLILGKLVKGLL